European Patent Application EP 4 631 975 A1, published October 15, 2025. Title: FUSION PROTEINS COMPRISING ANTI-TAU ANTIBODY AND PEPTIDE AND USES THEREOF. Applicant: 주식회사 아델. The sequence listing filed with the application follows.

SEQUENCE LISTING (39 sequences)

SEQ ID NO: 1 - DNA, 24 bp, synthetic construct
  source 1..24: mol_type = other DNA; note = nucleotide sequence for CDR1 of anti-tau antibody (VH)
ggagacagcatcacaagtggttac

SEQ ID NO: 2 - protein, 8 aa, synthetic construct
  source 1..8: note = amino acid seqeunce for CDR1 of anti-tau antibody (VH)
GDSITSGY

SEQ ID NO: 3 - DNA, 21 bp, synthetic construct
  source 1..21: mol_type = other DNA; note = nucleotide sequence for CDR2 of anti-tau antibody (VH)
atcagatattctggacgcaca

SEQ ID NO: 4 - protein, 7 aa, synthetic construct
  source 1..7: note = amino acid seqeunce for CDR2 of anti-tau antibody (VH)
IRYSGRT

SEQ ID NO: 5 - DNA, 21 bp, synthetic construct
  source 1..21: mol_type = other DNA; note = nucleotide sequence for CDR3 of anti-tau antibody (VH)
gcttctgtttatttcacttat

SEQ ID NO: 6 - protein, 7 aa, synthetic construct
  source 1..7: note = amino acid seqeunce for CDR3 of anti-tau antibody (VH)
ASVYFTY

SEQ ID NO: 7 - DNA, 339 bp, synthetic construct
  source 1..339: mol_type = other DNA; note = nucleotide seqeunce for VH-01 of anti-tau antibody
gaagtacaacttcaagagtctggccccggtctcgtcaagccctctcaaacactcagtttgacatgcaccgtatctggagacagcatcacaagtggttactggaactggattaggcagccacccggtaagggcttggaatatattggatatatcagatattctggacgcacatactataacccaagtcttaaatctagggtgaccataagcagagatacaagtaagaaccaattctctctcaagctttctagcgtcacagccgccgacactgcagtctattattgcgcttctgtttatttcacttattggggtcaaggaactctggtaaccgttagctca

SEQ ID NO: 8 - protein, 113 aa, synthetic construct
  source 1..113: note = amino acid seqeunce for VH-01 of anti-tau antibody
EVQLQESGPGLVKPSQTLSLTCTVSGDSITSGYWNWIRQPPGKGLEYIGYIRYSGRTYYNPSLKSRVTISRDTSKNQFSLKLSSVTAADTAVYYCASVYFTYWGQGTLVTVSS

SEQ ID NO: 9 - DNA, 33 bp, synthetic construct
  source 1..33: mol_type = other DNA; note = nucleotide sequence for CDR1 of anti-tau antibody (VL)
cagagcctgctggactccgacggcaagacctac

SEQ ID NO: 10 - protein, 11 aa, synthetic construct
  source 1..11: note = amino acid seqeunce for CDR1 of anti-tau antibody (VL)
QSLLDSDGKTY

SEQ ID NO: 11-12 - skipped (2 entries)

SEQ ID NO: 13 - DNA, 27 bp, synthetic construct
  source 1..27: mol_type = other DNA; note = nucleotide sequence for CDR3 of anti-tau antibody (VL)
tggcagggctctcacttcccctacacc

SEQ ID NO: 14 - protein, 9 aa, synthetic construct
  source 1..9: note = amino acid seqeunce for CDR3 of anti-tau antibody (VL)
WQGSHFPYT

SEQ ID NO: 15 - DNA, 336 bp, synthetic construct
  source 1..336: mol_type = other DNA; note = nucleotide seqeunce for VL-01 of anti-tau antibody
gacgttgtgatgacacaaagccctctgagcctgcctgtgacactgggacagcctgccagcatcagctgcaagtctagccagagcctgctggactccgacggcaagacctacctgaactggttccagcagaggcccggacagagccccaagagactgatcagcctggtgtccaagctggatagcggcgtgcccgatagattttctggctctggcagcggcaccgacttcaccctgaagatcagcagagtggaagccgaggacgtgggcgtgtactactgttggcagggctctcacttcccctacacctttggccagggcacaaagctggaaatcaag

SEQ ID NO: 16 - protein, 112 aa, synthetic construct
  source 1..112: note = amino acid seqeunce for VL-01 of anti-tau antibody
DVVMTQSPLSLPVTLGQPASISCKSSQSLLDSDGKTYLNWFQQRPGQSPKRLISLVSKLDSGVPDRFSGSGSGTDFTLKISRVEAEDVGVYYCWQGSHFPYTFGQGTKLEIK

SEQ ID NO: 17 - DNA, 60 bp, synthetic construct
  source 1..60: mol_type = other DNA; note = nucleotide seqeunce for linker
ggcggcggcggctctggaggaggaggcagcggcggcggcggctctggaggaggctccggc

SEQ ID NO: 18 - protein, 20 aa, synthetic construct
  source 1..20: note = amino acid seqeunce for linker
GGGGSGGGGSGGGGSGGGSG

SEQ ID NO: 19 - DNA, 57 bp, unidentified
  source 1..57: mol_type = other DNA; note = nucleotide sequence for APEP peptide
acttttttttatggtggttctcgtggtaaacgtaataattttaaaactgaagaatat

SEQ ID NO: 20 - protein, 19 aa, unidentified
  source 1..19: note = amino acid seqeunce for APEP peptide
TFFYGGSRGKRNNFKTEEY

SEQ ID NO: 21 - DNA, 87 bp, unidentified
  source 1..87: mol_type = other DNA; note = nucleotide sequence for RVG29 peptide
tacaccatctggatgccagagaacccccggcctggcaccccatgcgacatcttcacaaacagccggggcaagagagcctccaatggc

SEQ ID NO: 22 - protein, 29 aa, unidentified
  source 1..29: note = amino acid seqeunce for RVG29 peptide
YTIWMPENPRPGTPCDIFTNSRGKRASNG

SEQ ID NO: 23 - DNA, 36 bp, unidentified
  source 1..36: mol_type = other DNA; note = nucleotide sequence for TfR peptide
acccacaggccacctatgtggagcccagtgtggccc

SEQ ID NO: 24 - protein, 12 aa, unidentified
  source 1..12: note = amino acid seqeunce for TfR peptide
THRPPMWSPVWP

SEQ ID NO: 25 - protein, 441 aa, Homo sapiens
  source 1..441: note = Tau protein(WT)
MAEPRQEFEVMEDHAGTYGLGDRKDQGGYTMHQDQEGDTDAGLKESPLQTPTEDGSEEPGSETSDAKSTPTAEDVTAPLVDEGAPGKQAAAQPHTEIPEGTTAEEAGIGDTPSLEDEAAGHVTQARMVSKSKDGTGSDDKKAKGADGKTKIATPRGAAPPGQKGQANATRIPAKTPPAPKTPPSSGEPPKSGDRSGYSSPGSPGTPGSRSRTPSLPTPPTREPKKVAVVRTPPKSPSSAKSRLQTAPVPMPDLKNVKSKIGSTENLKHQPGGGKVQIINKKLDLSNVQSKCGSKDNIKHVPGGGSVQIVYKPVDLSKVTSKCGSLGNIHHKPGGGQVEVKSEKLDFKDRVQSKIGSLDNITHVPGGGNKKIETHKLTFRENAKAKTDHGAEIVYKSPVVSGDTSPRHLSNVSSTGSIDMVDSPQLATLADEVSASLAKQGL

SEQ ID NO: 26 - DNA, 339 bp, synthetic construct
  source 1..339: mol_type = other DNA; note = nucleotide seqeunce for VH-02 of anti-tau antibody
gaggtgcagctggaggagtcaggacctagcctcgtgaaaccttctcagactctgtccctcacctgttctgtcactggcgactccatcaccagtggttactggaactggatccggaaattcccagggaataaacttgagtacatggggtacataaggtacagtggtagaacttactacaatccatctctcaaaagtcgaatctccatcactcgagacacatcaaagaaccagttctacctgcagttgatttctgtgactactgaggacacagccacatattactgtgcaagtgtttactttacttactggggccaagggactctggtcactgtctctaca

SEQ ID NO: 27 - protein, 113 aa, synthetic construct
  source 1..113: note = amino acid seqeunce for VH-02 of anti-tau antibody
EVQLEESGPSLVKPSQTLSLTCSVTGDSITSGYWNWIRKFPGNKLEYMGYIRYSGRTYYNPSLKSRISITRDTSKNQFYLQLISVTTEDTATYYCASVYFTYWGQGTLVTVSS

SEQ ID NO: 28 - DNA, 339 bp, synthetic construct
  source 1..339: mol_type = other DNA; note = nucleotide seqeunce for VH-03 of anti-tau antibody
gaggtgcagctgcagcagagcggacccggactggtgaagcccagccagacactgtctttaacttgtgccgtgagcggcgatagcatcaccagcggctactggaactggattcgtcagagccctagcagaggtttagagtggctgggctacatcagatacagcggtcgtacctactacaacccctctttaaagtctcgtatcaccatcaatcgtgacaccagcaagaaccagttctctttacagctgaacagcgtgaccccagaagacaccgccgtgtactactgcgccagcgtgtacttcacctactggggccaaggtactttagtgaccgtctcgagc

SEQ ID NO: 29 - protein, 113 aa, synthetic construct
  source 1..113: note = amino acid seqeunce for VH-03 of anti-tau antibody
EVQLQQSGPGLVKPSQTLSLTCAVSGDSITSGYWNWIRQSPSRGLEWLGYIRYSGRTYYNPSLKSRITINRDTSKNQFSLQLNSVTPEDTAVYYCASVYFTYWGQGTLVTVSS

SEQ ID NO: 30 - DNA, 339 bp, synthetic construct
  source 1..339: mol_type = other DNA; note = nucleotide seqeunce for VH-04 of anti-tau antibody
gaggtgactttaaaggagagcggacccactttagtgaagcccacccagactttaactttaacttgtaccgtgagcggcgacagcatcaccagcggctactggaactggatcagacagccccccggcaaagctttagagtatttagcctacattcgttacagcggtcgtacatactacaacccctctttaaagtctcgtctgaccatcactcgtgacaccagcaagaaccaagttgtgctgaccatgaccaacatggaccccgtggacaccgccacctactactgcgccagcgtgtatttcacctactggggccaaggtactttagtgaccgtctcgagc

SEQ ID NO: 31 - protein, 113 aa, synthetic construct
  source 1..113: note = amino acid seqeunce for VH-04 of anti-tau antibody
EVTLKESGPTLVKPTQTLTLTCTVSGDSITSGYWNWIRQPPGKALEYLAYIRYSGRTYYNPSLKSRLTITRDTSKNQVVLTMTNMDPVDTATYYCASVYFTYWGQGTLVTVSS

SEQ ID NO: 32 - DNA, 339 bp, synthetic construct
  source 1..339: mol_type = other DNA; note = nucleotide seqeunce for VH-05 of anti-tau antibody
gaggtgcagctggtggagagcggcggaggactggtgcaacccggtcgttctttaaggctgagctgcaccgtgagcggcgacagcatcacctccggctactggaactggtttcgtcaagctcccggtaaaggtttagagtacgtgggctacattcgttacagcggtcgtacctactacaatccctctttaaagtctcgtttcaccatctctcgtgacaccagcaagaacatcgcctatttacagatgaactctttaaagaccgaggacaccgccgtgtactactgcgccagcgtgtacttcacctactggggccaaggtactttagtgaccgtctcgagc

SEQ ID NO: 33 - protein, 113 aa, synthetic construct
  source 1..113: note = amino acid seqeunce for VH-05 of anti-tau antibody
EVQLVESGGGLVQPGRSLRLSCTVSGDSITSGYWNWFRQAPGKGLEYVGYIRYSGRTYYNPSLKSRFTISRDTSKNIAYLQMNSLKTEDTAVYYCASVYFTYWGQGTLVTVSS

SEQ ID NO: 34 - DNA, 336 bp, synthetic construct
  source 1..336: mol_type = other DNA; note = nucleotide seqeunce for VL-02 of anti-tau antibody
gatgttttgatgacccaaactccactcactttgtcggttaccattggacaaccagcctccatctcttgcaagtcaagtcagagcctcttagatagtgatggaaagacatatttgaattggttgttacagaggccaggccagtctccaaagcgcctaatctctctggtgtctaagctggactctggagtccctgacaggttcactggcagtggatcagggacagatttcacactgaaaatcagccgagtggaggctgaggatttgggagtttattattgctggcaaggttcacattttccgtacacgttcggaggggggaccaagctggaaataaga

SEQ ID NO: 35 - protein, 112 aa, synthetic construct
  source 1..112: note = amino acid seqeunce for VL-02 of anti-tau antibody
DVLMTQTPLTLSVTIGQPASISCKSSQSLLDSDGKTYLNWLLQRPGQSPKRLISLVSKLDSGVPDRFTGSGSGTDFTLKISRVEAEDLGVYYCWQGSHFPYTFGGGTKLEIK

SEQ ID NO: 36 - DNA, 336 bp, synthetic construct
  source 1..336: mol_type = other DNA; note = nucleotide seqeunce for VL-03 of anti-tau antibody
gacgtggtgatgacacagagccccgattctttagctgtgtctttaggcgagagagccaccatcaactgcaagtccagccagtctttactggacagcgacggcaagacctatttaaactggtaccagcagaagcccggccagagccccaagaggctcatctctttagtgagcaagctggacagcggcgtgcccgataggttcagcggaagcggcagcggcaccgacttcactttaaccatcagctctttacaagctgaggatgtggccgtgtactactgctggcaaggtagccacttcccctacaccttcggccaaggtaccaagctcgagatcaag

SEQ ID NO: 37 - protein, 112 aa, synthetic construct
  source 1..112: note = amino acid seqeunce for VL-03 of anti-tau antibody
DVVMTQSPDSLAVSLGERATINCKSSQSLLDSDGKTYLNWYQQKPGQSPKRLISLVSKLDSGVPDRFSGSGSGTDFTLTISSLQAEDVAVYYCWQGSHFPYTFGQGTKLEIK

SEQ ID NO: 38 - DNA, 336 bp, synthetic construct
  source 1..336: mol_type = other DNA; note = nucleotide seqeunce for VL-04 of anti-tau antibody
gaggtggtgctgacccagagccccggtactttatctttaagccccggtgagagagccactttaagctgcaagagcagccagtctttactggacagcgacggcaagacctatttaaactggtaccagcagaagcccggccagagccccaagaggctgatctctttagtgagcaagctggacagcggcatccccgacagattcagcggaagcggcagcggcaccgacttcactttaaccatctctcgtctggagccagaagacttcgccgtgtactactgctggcaaggtagccacttcccctacaccttcggccaaggtaccaagctcgagatcaag

SEQ ID NO: 39 - protein, 112 aa, synthetic construct
  source 1..112: note = amino acid seqeunce for VL-04 of anti-tau antibody
EVVLTQSPGTLSLSPGERATLSCKSSQSLLDSDGKTYLNWYQQKPGQSPKRLISLVSKLDSGIPDRFSGSGSGTDFTLTISRLEPEDFAVYYCWQGSHFPYTFGQGTKLEIK